European Patent Application EP 4 137 515 A1, published February 22, 2023. Title: ANTIGEN-BINDING POLYPEPTIDES AGAINST CD73. Applicant: Universitätsklinikum Hamburg-Eppendorf. The sequence listing filed with the application follows.

SEQUENCE LISTING (84 sequences)

SEQ ID NO: 1 - protein, 9 aa, Vicugna pacos
  consensus sequence CDR1 - Family 1
  SITE 4: Xaa = Thr or Ala
  SITE 8: Xaa = Leu or Tyr
  SITE 9: Xaa = Ser or Thr
SGFXLDYXX

SEQ ID NO: 2 - protein, 7 aa, Vicugna pacos
  SITE 1: Xaa = Ile or Val
  consensus sequence CDR2 - Family 1
  SITE 2: Xaa = Ser or Asn
  SITE 4: Xaa = Ser or Asn
  SITE 6: Xaa = Gly, Ser or Asp
  SITE 7: Xaa = Ser, Ile, Val or Arg
XXSXGXX

SEQ ID NO: 3 - protein, 15 aa, Vicugna pacos
  SITE 1: Xaa = His or Gln
  consensus sequence CDR3 - Family 1
  SITE 2: Xaa = Lys or Arg
  SITE 8: Xaa = Asn, Gly, Arg or Asp
  SITE 9: Xaa = Lys or Arg
  SITE 10: Xaa = Gly, Ala or Val
  SITE 11: Xaa = Glu or Ala
  SITE 13: Xaa = Phe or Tyr
  SITE 15: Xaa = Tyr or Ser
XXYYYCSXXXXVXDX

SEQ ID NO: 4 - protein, 9 aa, Vicugna pacos
  CDR1 of clone SB96
SGFTLDYLS

SEQ ID NO: 5 - protein, 7 aa, Vicugna pacos
  CDR2 of clone SB96
INSSGGS

SEQ ID NO: 6 - protein, 15 aa, Vicugna pacos
  CDR3 of clone SB96
HKYYYCSNKVEVFDY

SEQ ID NO: 7 - protein, 9 aa, Vicugna pacos
  CDR1 of clone SB98
SGFTLDYYT

SEQ ID NO: 8 - protein, 7 aa, Vicugna pacos
  CDR2 of clone SB98
ISSSGGI

SEQ ID NO: 9 - protein, 15 aa, Vicugna pacos
  CDR3 of clone SB98
QKYYYCSGKAEVYDY

SEQ ID NO: 10 - protein, 9 aa, Vicugna pacos
  CDR1 of clone SB115
SGFTLDYYT

SEQ ID NO: 11 - protein, 7 aa, Vicugna pacos
  CDR2 of clone SB115
INSSGGV

SEQ ID NO: 12 - protein, 15 aa, Vicugna pacos
  CDR3 of clone SB115
QKYYYCSRKGEVYDS

SEQ ID NO: 13 - protein, 9 aa, Vicugna pacos
  CDR1 of clone SB123
SGFTLDYLS

SEQ ID NO: 14 - protein, 7 aa, Vicugna pacos
  CDR2 of clone SB123
INSSGGS

SEQ ID NO: 15 - protein, 15 aa, Vicugna pacos
  CDR3 of clone SB123
HKYYYCSNKVAVFDY

SEQ ID NO: 16 - protein, 9 aa, Vicugna pacos
  CDR1 of clone SB124
SGFTLDYYT

SEQ ID NO: 17 - protein, 7 aa, Vicugna pacos
  CDR2 of clone SB124
VSSSGDR

SEQ ID NO: 18 - protein, 15 aa, Vicugna pacos
  CDR3 of clone SB124
QKYYYCSGKVEVYDY

SEQ ID NO: 19 - protein, 9 aa, Vicugna pacos
  CDR1 of clone SB107
SGFTLDYLT

SEQ ID NO: 20 - protein, 7 aa, Vicugna pacos
  CDR2 of clone SB107
INSNGGS

SEQ ID NO: 21 - protein, 15 aa, Vicugna pacos
  CDR3 of clone SB107
QKYYYCSGRVEVYDY

SEQ ID NO: 22 - protein, 9 aa, Vicugna pacos
  CDR1 of clone SB108
SGFALDYYT

SEQ ID NO: 23 - protein, 7 aa, Vicugna pacos
  CDR2 of clone SB108
ISSSGSS

SEQ ID NO: 24 - protein, 15 aa, Vicugna pacos
  CDR3 of clone SB108
QRYYYCSDKVAVYDY

SEQ ID NO: 25 - protein, 9 aa, Vicugna pacos
  CDR1 of clone SB125
SGFALDYYT

SEQ ID NO: 26 - protein, 7 aa, Vicugna pacos
  CDR2 of clone SB125
ISSSGGS

SEQ ID NO: 27 - protein, 15 aa, Vicugna pacos
  CDR3 of clone SB125
QRYYYCSDKVEVYDY

SEQ ID NO: 28 - protein, 9 aa, Vicugna pacos
  consensus sequence CDR1 - Family 2
  SITE 7: Xaa = Arg or Gly
SGRTFSXST

SEQ ID NO: 29 - protein, 7 aa, Vicugna pacos
  consensus sequence CDR2 - Family 2
IRWIGGT

SEQ ID NO: 30 - protein, 17 aa, Vicugna pacos
  consensus sequence CDR3 - Family 2
  SITE 6: Xaa = Tyr or Asp
  SITE 13: Xaa = Ile or Thr
  SITE 14: Xaa = Leu or Val
TAGGPXYLGGRDXXYDY

SEQ ID NO: 31 - protein, 9 aa, Vicugna pacos
  CDR1 of clone SB143
SGRTFSRST

SEQ ID NO: 32 - protein, 7 aa, Vicugna pacos
  CDR2 of clone SB143
IRWIGGT

SEQ ID NO: 33 - protein, 17 aa, Vicugna pacos
  CDR3 of clone SB143
TAGGPYYLGGRDILYDY

SEQ ID NO: 34 - protein, 9 aa, Vicugna pacos
  CDR1 of clone SB144
SGRTFSGST

SEQ ID NO: 35 - protein, 7 aa, Vicugna pacos
  CDR2 of clone SB144
IRWIGGT

SEQ ID NO: 36 - protein, 17 aa, Vicugna pacos
  CDR3 of clone SB144
TAGGPDYLGGRDIVYDY

SEQ ID NO: 37 - protein, 9 aa, Vicugna pacos
  CDR1 of clone SB151
SGRTFSRST

SEQ ID NO: 38 - protein, 7 aa, Vicugna pacos
  CDR2 of clone SB151
IRWIGGT

SEQ ID NO: 39 - protein, 17 aa, Vicugna pacos
  CDR3 of clone SB151
TAGGPDYLGGRDTLYDY

SEQ ID NO: 40 - protein, 9 aa, Vicugna pacos
  consensus sequence CDR1 - Family 3
  SITE 6: Xaa = Ile or Thr
SGFTFXNYH

SEQ ID NO: 41 - protein, 7 aa, Vicugna pacos
  consensus sequence CDR2 - Family 3
IHSRGDI

SEQ ID NO: 42 - protein, 12 aa, Vicugna pacos
  consensus sequence CDR3 - Family 3
  SITE 6: Xaa = Gly or Asn
SRDLFXEGEYDY

SEQ ID NO: 43 - protein, 9 aa, Vicugna pacos
  CDR1 of clone SB141
SGFTFINYH

SEQ ID NO: 44 - protein, 7 aa, Vicugna pacos
  CDR2 of clone SB141
IHSRGDI

SEQ ID NO: 45 - protein, 12 aa, Vicugna pacos
  CDR3 of clone SB141
SRDLFNEGEYDY

SEQ ID NO: 46 - protein, 9 aa, Vicugna pacos
  CDR1 of clone SB142
SGFTFINYH

SEQ ID NO: 47 - protein, 7 aa, Vicugna pacos
  CDR2 of clone SB142
IHSRGDI

SEQ ID NO: 48 - protein, 12 aa, Vicugna pacos
  CDR3 of clone SB142
SRDLFGEGEYDY

SEQ ID NO: 49 - protein, 9 aa, Vicugna pacos
  CDR1 of clone SB148
SGFTFTNYH

SEQ ID NO: 50 - protein, 7 aa, Vicugna pacos
  CDR2 of clone SB148
IHSRGDI

SEQ ID NO: 51 - protein, 12 aa, Vicugna pacos
  CDR3 of clone SB148
SRDLFNEGEYDY

SEQ ID NO: 52 - protein, 9 aa, Vicugna pacos
  CDR1 of clone SB167
SGFTFINYH

SEQ ID NO: 53 - protein, 7 aa, Vicugna pacos
  CDR2 of clone SB167
IHSRGDI

SEQ ID NO: 54 - protein, 12 aa, Vicugna pacos
  CDR3 of clone SB167
SRDLFGEGEYDY

SEQ ID NO: 55 - protein, 9 aa, Vicugna pacos
  CDR1 of clone SB188
SGFTFINYH

SEQ ID NO: 56 - protein, 7 aa, Vicugna pacos
  CDR2 of clone SB188
IHSRGDI

SEQ ID NO: 57 - protein, 12 aa, Vicugna pacos
  CDR3 of clone SB188
SRDLFNEGEYDY

SEQ ID NO: 58 - protein, 9 aa, Vicugna pacos
  CDR1 of clone SB189
SGFTFTNYH

SEQ ID NO: 59 - protein, 7 aa, Vicugna pacos
  CDR2 of clone SB189
IHSRGDI

SEQ ID NO: 60 - protein, 12 aa, Vicugna pacos
  CDR3 of clone SB189
SRDLFNEGEYDY

SEQ ID NO: 61 - protein, 124 aa, Vicugna pacos
  clone SB96
DVQLQASGGGLVQPGGSLRLSCTASGFTLDYLSIGWFRQVPGKEREGVSCINSSGGSTNYADSLKGRLTISRDNAKNTVYLQMNSLKPEDTAVYYCAAHKYYYCSNKVEVFDYWGQGTPVTVSS

SEQ ID NO: 62 - protein, 124 aa, Vicugna pacos
  clone SB98
QVKLQESGGGLVQPGGSLRLSCAASGFTLDYYTIGWFRQAPGKEREGVSCISSSGGITNYADSVKGRLTISRDNAKNTVYLQMNSLKPEDTAVYYCAAQKYYYCSGKAEVYDYWGQGTQVTVSS

SEQ ID NO: 63 - protein, 124 aa, Vicugna pacos
  clone SB115
DVQLQASGGGLVQPGGSLRLSCVVSGFTLDYYTIGWFRQAPGKEREGVSCINSSGGVTNYADSVKGRFTISRDNAKNTVYLQMNSLKSEDTAVYYCAAQKYYYCSRKGEVYDSWGQGTQVTVSS

SEQ ID NO: 64 - protein, 124 aa, Vicugna pacos
  clone SB123
DVQLQESGGGLVQPGGSLTLSCAASGFTLDYLSIGWFRQVPGKEREGVSCINSSGGSTNYADSVKGRLTISRDNAKNTVYLQINSLKPEDTAVYYCAAHKYYYCSNKVAVFDYWGQGTQVTVSS

SEQ ID NO: 65 - protein, 124 aa, Vicugna pacos
  clone SB124
QVQLQESGGGLVQPGGSLRLSCAASGFTLDYYTIGWFRQAPGKEREGVSCVSSSGDRTDYLESVKGRLTISRDNAKNTVYLQMNSLKPEDTGVYYCAAQKYYYCSGKVEVYDYWGQGTQVTVSS

SEQ ID NO: 66 - protein, 124 aa, Vicugna pacos
  clone SB107
QVQLQESGGGLVQPGGSLRLSCAASGFTLDYLTIGWFRQAPGKEREGVSCINSNGGSTIYADSVKGRLTISRDNAKNTVYLQINSLKPDDTAVYFCAAQKYYYCSGRVEVYDYWGQGIQVTVSS

SEQ ID NO: 67 - protein, 124 aa, Vicugna pacos
  clone SB108
QVKLQESGGGLVHSGGSLRLSCAVSGFALDYYTIGWFRQAPGKEREGVSCISSSGSSTNYADSMKGRLTISRDNAKNTVYLQMNSLKPEDTAVYYCAAQRYYYCSDKVAVYDYWGQGTQVTVSS

SEQ ID NO: 68 - protein, 124 aa, Vicugna pacos
  clone SB125
QVQLQESGGGLVQPGGSLRLSCAVSGFALDYYTIGWFRQAPGKEREGVSCISSSGGSTNYADSVKGRLTISRDNAKNTVYLQMNSLKPEDTAVYYCAAQRYYYCSDKVEVYDYWGQGTQVTVSS

SEQ ID NO: 69 - protein, 126 aa, Vicugna pacos
  clone SB143
QVQLVESGGGLVQAGGSLRLSCAASGRTFSRSTMGWFRQAPGKERVFVAAIRWIGGTTTYGDSVKGRFTISVDNAKNTLYLQMNSLKPEDTAVYYCAATAGGPYYLGGRDILYDYWGQGTQVTVSS

SEQ ID NO: 70 - protein, 126 aa, Vicugna pacos
  clone SB144
QVQLVESGGGLVQAGGSLRLSCAASGRTFSGSTMGWFRQAPGKERAFVAAIRWIGGTAKYGDSVKGRFTISIDNAKNTLYLQMNSLKPEDTAVYYCAATAGGPDYLGGRDIVYDYWGQGTQVTVSS

SEQ ID NO: 71 - protein, 126 aa, Vicugna pacos
  clone SB151
QVQLVESGGGLVQAGGSLRLSCAASGRTFSRSTMGWFRQAPGKERVFVAAIRWIGGTTNYGDSVKGRFTISVDNAKNTLYLQMNSLKPEDTAVYYCAATAGGPDYLGGRDTLYDYWGQGTQVTVSS

SEQ ID NO: 72 - protein, 121 aa, Vicugna pacos
  clone SB141
QVQLVESGGGLVQPGGSLRLSCAASGFTFINYHMSWLRQAPGKGLEWVSEIHSRGDITSYTNSVKGRFTISRDNAKNTLYLQMNSLKFDDTAVYYCARSRDLFNEGEYDYWGRGTQVTVSS

SEQ ID NO: 73 - protein, 121 aa, Vicugna pacos
  clone SB142
QVQLVESGGGLVQPGGSLRLSCAASGFTFINYHMSWLRQAPGKGLEWVSEIHSRGDITSYTNSVKGRFTISRDNAKNTLYLQMNSLKFDDTAVYYCARSRDLFGEGEYDYWGRGTQVTVSS

SEQ ID NO: 74 - protein, 121 aa, Vicugna pacos
  clone SB148
QVQLVESGGGLVQPGGSLRLSCAASGFTFTNYHMSWLRQAPGKGLEWVSEIHSRGDITSYTNSVKGRFTISRDNAKNMLYLQMNSLKFDDTAVYYCARSRDLFNEGEYDYWGRGTQVTVSS

SEQ ID NO: 75 - protein, 121 aa, Artificial Sequence
  clone derived by CDR grafting
QVQLVESGGGLVQAGGSLRLSCAASGFTFINYHMSWLRQAPGKEREFVAEIHSRGDITSYTNSVKGRFTISRDNAKNTVYLQMNSLKPEDTAVYYCARSRDLFGEGEYDYWGRGTQVTVSS

SEQ ID NO: 76 - protein, 121 aa, Artificial Sequence
  clone derived by CDR grafting
QVQLVESGGGLVQAGGSLRLSCAASGFTFINYHMSWLRQAPGKEREFVAEIHSRGDITSYTNSVKGRFTISRDNAKNTVYLQMNSLKPEDTAVYYCARSRDLFNEGEYDYWGRGTQVTVSS

SEQ ID NO: 77 - protein, 121 aa, Artificial Sequence
  clone derived by CDR grafting
QVQLVESGGGLVQAGGSLRLSCAASGFTFTNYHMSWLRQAPGKEREFVAEIHSRGDITSYTNSVKGRFTISRDNAKNMVYLQMNSLKPEDTAVYYCARSRDLFNEGEYDYWGRGTQVTVSS

SEQ ID NO: 78 - protein, 9 aa, Vicugna pacos
  CDR1 of clone SB116
SGISFSITT

SEQ ID NO: 79 - protein, 6 aa, Vicugna pacos
  CDR2 of clone SB116
ITDRGN

SEQ ID NO: 80 - protein, 5 aa, Vicugna pacos
  CDR3 of clone SB116
IPGND

SEQ ID NO: 81 - protein, 113 aa, Vicugna pacos
  clone SB116
QVKLQESGGGRVQTGGSLRLSCAASGISFSITTMYWYRQAPGEQRQLVALITDRGNTYYVDSVKGRFTISRDDSKNTVYLQMNDLKPEDTAVYFCNSIPGNDWGQGTQVTVSS

SEQ ID NO: 82 - protein, 116 aa, Vicugna pacos
  clone SB121
QVQLQESGGGLVQAGGSLRLSCAASGSIGSIIAMGWYRQGPGKQRELVARMFTDDGSTNYDDSVKGRFTISRDSAGTTVYLQMNSLKPEDTAVYYCNAQRRWNAYWGPGTQVTVSS

SEQ ID NO: 83 - protein, 111 aa, Vicugna pacos
  clone SB139
QVQLQESGGGLVQAGGSLRLSCAASENIFNIYGMGWYRQAPGKLRDLVAKITSGGRTTYADSVKGRFTISGDNAKNTVYLQMNSLKPEDTAVYYCNSYYYWGQGTQVTVSS

SEQ ID NO: 84 - protein, 574 aa, Homo sapiens
  CD73
MCPRAARAPATLLLALGAVLWPAAGAWELTILHTNDVHSRLEQTSEDSSKCVNASRCMGGVARLFTKVQQIRRAEPNVLLLDAGDQYQGTIWFTVYKGAEVAHFMNALRYDAMALGNHEFDNGVEGLIEPLLKEAKFPILSANIKAKGPLASQISGLYLPYKVLPVGDEVVGIVGYTSKETPFLSNPGTNLVFEDEITALQPEVDKLKTLNVNKIIALGHSGFEMDKLIAQKVRGVDVVVGGHSNTFLYTGNPPSKEVPAGKYPFIVTSDDGRKVPVVQAYAFGKYLGYLKIEFDERGNVISSHGNPILLNSSIPEDPSIKADINKWRIKLDNYSTQELGKTIVYLDGSSQSCRFRECNMGNLICDAMINNNLRHTDEMFWNHVSMCILNGGGIRSPIDERNNGTITWENLAAVLPFGGTFDLVQLKGSTLKKAFEHSVHRYGQSTGEFLQVGGIHVVYDLSRKPGDRVVKLDVLCTKCRVPSYDPLKMDEVYKVILPNFLANGGDGFQMIKDELLRHDSGDQDINVVSTYISKMKVIYPAVEGRIKFSTGSHCHGSFSLIFLSLWAVIFVLYQ